European Patent Application EP 4 317 438 A1, published February 7, 2024. Title: Recombinant polypeptide with acyl-CoA compound reducing activity. Applicant: Asahi Kasei Corporation. The sequence listing filed with the application follows.

SEQUENCE LISTING (157 sequences)

SEQ ID NO: 1 - protein, 463 aa, Clostridium difficile
MEKAVENFEDLSKEYINGYIERARKAQREFECYTQEQVDKIVKIVGKVVYYNAEYLAKLAVEETGMGVYEDKVAKNKSKAKVIYNNLKDKKSVGIIDIDRETGITKVAKPVGVVAAITPCTNPIVTPMSNAMFALKGRNAIIITPHHKAIGCSTKTVEMINEELEKIGAPENLIQILDQQSRENTRNLISSADVVIATGGMGMVKAAYSSGKPALGVGAGNVQCIIDRDVDIKEAVPKIIAGRIFDNGIICSGEQSVIVAEEMFDKIMDEFKNNKGFIVRDKVQKEAFRNAMFVNKSMNKDAVGQSVHTIAKIAGVEIPEDTKIIVIEADGPGEEDIIAKEKMCPVISAYKYKSFEEGVAIAKANLNVEGKGHSVSIHSNTVKNIEYAGENIEVSRFVINQCCATSAGGSFFNGLAPTNTLGCGSWGNNSISENLDYKHLINISRIAYYMPENEVPTDEELWG

SEQ ID NO: 2 - DNA, 1389 bp, Clostridium difficile
atggaaaaagcagtggaaaactttgaagatttaagtaaggaatacattaatggttatattgagagagcaagaaaagctcaaagagagtttgaatgttatactcaagaacaagtagataaaatagtaaaaatagttggaaaagtagtgtattataatgctgaatatttagctaaacttgctgtagaagagactggaatgggagtatatgaagataaggtagctaaaaataaaagcaaagcaaaagttatatataacaatttaaaagataaaaaatcagttggtataattgatatagatagagaaactggaataacaaaggtagctaaaccagttggagtagtagcggcaataactccttgtacaaatccaatcgttacacctatgagcaatgcaatgtttgcacttaagggaagaaatgcaattattatcacacctcatcataaagcaattggatgtagtacaaaaactgtagagatgattaatgaagaattagaaaaaataggagctccagaaaatttaatacaaatacttgaccaacaatcaagagaaaatacaagaaatttaatttcatcagcagatgtagtaattgccactggaggaatgggaatggtaaaagctgcgtactcaagtggaaaaccagcacttggtgtaggggcaggaaatgttcaatgtatcatagatagagatgtagacattaaagaagcagtacctaaaatcatagcaggaagaatttttgataatggtatcatttgttcaggtgaacagtcagtaatagtagcagaagaaatgtttgataaaataatggatgaatttaaaaataataaaggttttatagttagagataaagtacaaaaagaagctttcagaaatgctatgtttgtaaataaatctatgaataaagatgcagtaggtcaatcagttcatacaattgcaaaaattgcaggtgttgagataccagaagatacaaaaataatagtaatagaagctgatggaccaggagaagaggatattattgcaaaagaaaaaatgtgtccagttatatctgcatacaagtataaaagttttgaagaaggtgtagctattgcaaaagcaaatttaaatgtagaaggaaaaggacatagtgtatctatacattcaaatacagttaaaaatatagaatatgcaggagaaaatatagaagtatcaagatttgttattaatcaatgttgtgctactagtgctggaggaagtttctttaatggtcttgcacctactaatactctaggttgtggttcttggggaaataacagcatctctgaaaatcttgattataagcatctaattaatatttctagaattgcttattatatgccagaaaatgaagtccctacagatgaagaactttgggga

SEQ ID NO: 3 - DNA, 155 bp, Artificial Sequence
  promoter
ctcaagcccaaaggaagagtgaggcgagtcagtcgcgtaatgcttaggcacaggattgatttgtcgcaatgattgacacgattccgcttgacgctgcgtaaggtttttgtaattttacaggcaaccttttattcactaacaaatagctggtggaa

SEQ ID NO: 4 - DNA, 47 bp, Artificial Sequence
  terminator
aaaaaaaaaaaggtgccgtggaaacacggcacctttttttttcttta

SEQ ID NO: 5 - DNA, 21 bp, Artificial Sequence
  primer 1
atggaaaaagcagtcgagaac

SEQ ID NO: 6 - DNA, 21 bp, Artificial Sequence
  primer 2
ttagccccataattcttcgtc

SEQ ID NO: 7 - DNA, 20 bp, Artificial Sequence
  primer 3
atgatacgcgagcctccgga

SEQ ID NO: 8 - DNA, 21 bp, Artificial Sequence
  primer 4
ttacgcttcttcgacacttac

SEQ ID NO: 9 - DNA, 24 bp, Artificial Sequence
  primer 5
atgtcgatgataaaaagctatgcc

SEQ ID NO: 10 - DNA, 22 bp, Artificial Sequence
  primer 6
tcaaaaatcggctttcaacacc

SEQ ID NO: 11 - DNA, 35 bp, Artificial Sequence
  fw primer
tttaaaaacaaaagcaaagccaaagtcatctacaa

SEQ ID NO: 12 - DNA, 30 bp, Artificial Sequence
  rv primer
aactttgtcttcatagactcccatacccgt

SEQ ID NO: 13 - DNA, 30 bp, Artificial Sequence
  fw primer
cgtaaaaacaaaagcaaagccaaagtcatc

SEQ ID NO: 14 - DNA, 30 bp, Artificial Sequence; identical to SEQ ID NO: 12
  rv primer

SEQ ID NO: 15 - DNA, 32 bp, Artificial Sequence
  fw primer
gctaacaaaagcaaagccaaagtcatctacaa

SEQ ID NO: 16 - DNA, 30 bp, Artificial Sequence
  rv primer
agcaactttgtcttcatagactcccatacc

SEQ ID NO: 17 - DNA, 32 bp, Artificial Sequence
  fw primer
tttaacaaaagcaaagccaaagtcatctacaa

SEQ ID NO: 18 - DNA, 30 bp, Artificial Sequence; identical to SEQ ID NO: 16
  rv primer

SEQ ID NO: 19 - DNA, 32 bp, Artificial Sequence
  fw primer
gctaaagccaaagtcatctacaacaatctgaa

SEQ ID NO: 20 - DNA, 33 bp, Artificial Sequence
  rv primer
tttgtttttagcaactttgtcttcatagactcc

SEQ ID NO: 21 - DNA, 35 bp, Artificial Sequence
  fw primer
tttaaagccaaagtcatctacaacaatctgaagga

SEQ ID NO: 22 - DNA, 33 bp, Artificial Sequence; identical to SEQ ID NO: 20
  rv primer

SEQ ID NO: 23 - DNA, 31 bp, Artificial Sequence
  fw primer
gctgccaaagtcatctacaacaatctgaagg

SEQ ID NO: 24 - DNA, 33 bp, Artificial Sequence
  rv primer
gcttttgtttttagcaactttgtcttcatagac

SEQ ID NO: 25 - DNA, 31 bp, Artificial Sequence
  fw primer
tttgccaaagtcatctacaacaatctgaagg

SEQ ID NO: 26 - DNA, 33 bp, Artificial Sequence; identical to SEQ ID NO: 24
  rv primer

SEQ ID NO: 27 - DNA, 27 bp, Artificial Sequence
  fw primer
gctgataatgggatcatttgctctggc

SEQ ID NO: 28 - DNA, 24 bp, Artificial Sequence
  rv primer
aatgcgcccggcaataatctttgg

SEQ ID NO: 29 - DNA, 27 bp, Artificial Sequence
  fw primer
cgtgataatgggatcatttgctctggc

SEQ ID NO: 30 - DNA, 24 bp, Artificial Sequence
  rv primer
aatgcgcccggcaataatctttgg

SEQ ID NO: 31 - DNA, 24 bp, Artificial Sequence
  fw primer
gcttttttcaatggcttagcgccc

SEQ ID NO: 32 - DNA, 18 bp, Artificial Sequence
  rv primer
gccacctgcagacgtcgc

SEQ ID NO: 33 - DNA, 27 bp, Artificial Sequence
  fw primer
ttttttttcaatggcttagcgcccacg

SEQ ID NO: 34 - DNA, 18 bp, Artificial Sequence
  rv primer
gccacctgcagacgtcgc

SEQ ID NO: 35 - DNA, 23 bp, Artificial Sequence
  fw primer
gctttcaatggcttagcgcccac

SEQ ID NO: 36 - DNA, 21 bp, Artificial Sequence
  rv primer
gctgccacctgcagacgtcgc

SEQ ID NO: 37 - DNA, 23 bp, Artificial Sequence
  fw primer
cgtttcaatggcttagcgcccac

SEQ ID NO: 38 - DNA, 21 bp, Artificial Sequence
  rv primer
gctgccacctgcagacgtcgc

SEQ ID NO: 39 - DNA, 28 bp, Artificial Sequence
  fw primer
ttctgctctggcgaacagagtgtcattg

SEQ ID NO: 40 - DNA, 27 bp, Artificial Sequence
  rv primer
gatcccattatcaaaaatgcgcccggc

SEQ ID NO: 41 - DNA, 28 bp, Artificial Sequence
  fw primer
gcgtgctctggcgaacagagtgtcattg

SEQ ID NO: 42 - DNA, 27 bp, Artificial Sequence
  rv primer
gatcccattatcaaaaatgcgcccggc

SEQ ID NO: 43 - DNA, 29 bp, Artificial Sequence
  fw primer
ttttctggcgaacagagtgtcattgtggc

SEQ ID NO: 44 - DNA, 30 bp, Artificial Sequence
  rv primer
aatgatcccattatcaaaaatgcgcccggc

SEQ ID NO: 45 - DNA, 28 bp, Artificial Sequence
  fw primer
tttggcgaacagagtgtcattgtggcgg

SEQ ID NO: 46 - DNA, 31 bp, Artificial Sequence
  rv primer
gcaaatgatcccattatcaaaaatgcgcccg

SEQ ID NO: 47 - DNA, 28 bp, Artificial Sequence
  fw primer
gcgggcgaacagagtgtcattgtggcgg

SEQ ID NO: 48 - DNA, 31 bp, Artificial Sequence; identical to SEQ ID NO: 46
  rv primer

SEQ ID NO: 49 - DNA, 28 bp, Artificial Sequence
  fw primer
tttacgtctgcaggtggcagctttttca

SEQ ID NO: 50 - DNA, 31 bp, Artificial Sequence
  rv primer
acagcactgattgatcacaaaacgagacacc

SEQ ID NO: 51 - DNA, 34 bp, Artificial Sequence
  fw primer
ttttctgcaggtggcagctttttcaatggcttag

SEQ ID NO: 52 - DNA, 29 bp, Artificial Sequence
  rv primer
cgcacagcactgattgatcacaaaacgag

SEQ ID NO: 53 - DNA, 34 bp, Artificial Sequence
  fw primer
gcgtctgcaggtggcagctttttcaatggcttag

SEQ ID NO: 54 - DNA, 29 bp, Artificial Sequence
  rv primer
cgcacagcactgattgatcacaaaacgag

SEQ ID NO: 55 - DNA, 32 bp, Artificial Sequence
  fw primer
tttgcaggtggcagctttttcaatggcttagc

SEQ ID NO: 56 - DNA, 29 bp, Artificial Sequence
  rv primer
cgtcgcacagcactgattgatcacaaaac

SEQ ID NO: 57 - DNA, 32 bp, Artificial Sequence
  fw primer
gcggcaggtggcagctttttcaatggcttagc

SEQ ID NO: 58 - DNA, 29 bp, Artificial Sequence
  rv primer
cgtcgcacagcactgattgatcacaaaac

SEQ ID NO: 59 - DNA, 31 bp, Artificial Sequence
  fw primer
tttggtggcagctttttcaatggcttagcgc

SEQ ID NO: 60 - DNA, 27 bp, Artificial Sequence
  rv primer
agacgtcgcacagcactgattgatcac

SEQ ID NO: 61 - DNA, 30 bp, Artificial Sequence
  fw primer
tttggcagctttttcaatggcttagcgccc

SEQ ID NO: 62 - DNA, 28 bp, Artificial Sequence
  rv primer
tgcagacgtcgcacagcactgattgatc

SEQ ID NO: 63 - DNA, 30 bp, Artificial Sequence
  fw primer
tttagctttttcaatggcttagcgcccacg

SEQ ID NO: 64 - DNA, 24 bp, Artificial Sequence
  rv primer
acctgcagacgtcgcacagcactg

SEQ ID NO: 65 - DNA, 28 bp, Artificial Sequence
  fw primer
tttaataccttgggctgtggctcatggg

SEQ ID NO: 66 - DNA, 27 bp, Artificial Sequence
  rv primer
gggcgctaagccattgaaaaagctgcc

SEQ ID NO: 67 - DNA, 28 bp, Artificial Sequence
  fw primer
gcgaataccttgggctgtggctcatggg

SEQ ID NO: 68 - DNA, 27 bp, Artificial Sequence
  rv primer
gggcgctaagccattgaaaaagctgcc

SEQ ID NO: 69 - DNA, 25 bp, Artificial Sequence
  fw primer
tttaccttgggctgtggctcatggg

SEQ ID NO: 70 - DNA, 26 bp, Artificial Sequence
  rv primer
cgtgggcgctaagccattgaaaaagc

SEQ ID NO: 71 - DNA, 25 bp, Artificial Sequence
  fw primer
gcgaccttgggctgtggctcatggg

SEQ ID NO: 72 - DNA, 26 bp, Artificial Sequence
  rv primer
cgtgggcgctaagccattgaaaaagc

SEQ ID NO: 73 - DNA, 24 bp, Artificial Sequence
  fw primer
ttcttgggctgtggctcatggggc

SEQ ID NO: 74 - DNA, 28 bp, Artificial Sequence
  rv primer
attcgtgggcgctaagccattgaaaaag

SEQ ID NO: 75 - DNA, 24 bp, Artificial Sequence
  fw primer
gcgttgggctgtggctcatggggc

SEQ ID NO: 76 - DNA, 28 bp, Artificial Sequence
  rv primer
attcgtgggcgctaagccattgaaaaag

SEQ ID NO: 77 - DNA, 36 bp, Artificial Sequence
  fw primer
ttgttgaataaatcgtctgtttgccgagaatacgcg

SEQ ID NO: 78 - DNA, 35 bp, Artificial Sequence
  rv primer
tatcgcatgcagatctgcgctaatgggctccagga

SEQ ID NO: 79 - DNA, 35 bp, Artificial Sequence
  fw primer
ttgttgaataaatcgcgcgccagcgctggctgttt

SEQ ID NO: 80 - DNA, 35 bp, Artificial Sequence
  rv primer
tatcgcatgcagatcccgccaatgccggaagagtt

SEQ ID NO: 81 - DNA, 35 bp, Artificial Sequence
  fw primer
ttgttgaataaatcgcgatcgtgatgccgctgtct

SEQ ID NO: 82 - DNA, 35 bp, Artificial Sequence
  rv primer
tatcgcatgcagatcgacaacgtaggctttgttca

SEQ ID NO: 83 - DNA, 35 bp, Artificial Sequence
  fw primer
ttgttgaataaatcgcgccatctcgacactcttga

SEQ ID NO: 84 - DNA, 35 bp, Artificial Sequence
  rv primer
tatcgcatgcagatcgcgaacatcgatgggttagc

SEQ ID NO: 85 - DNA, 35 bp, Artificial Sequence
  fw primer
ttgttgaataaatcgtggcatttgcccttcctgtt

SEQ ID NO: 86 - DNA, 35 bp, Artificial Sequence
  rv primer
tatcgcatgcagatcgtcctgatcctgcaacggaa

SEQ ID NO: 87 - DNA, 35 bp, Artificial Sequence
  fw primer
ttgttgaataaatcgctcataacggtactgcaaac

SEQ ID NO: 88 - DNA, 35 bp, Artificial Sequence
  rv primer
tatcgcatgcagatctcgcagcaggtaagatgatt

SEQ ID NO: 89 - DNA, 35 bp, Artificial Sequence
  fw primer
ttgttgaataaatcgatattcgtcctaacgaacag

SEQ ID NO: 90 - DNA, 35 bp, Artificial Sequence
  rv primer
tatcgcatgcagatctttttgattttcaagtatgt

SEQ ID NO: 91 - DNA, 35 bp, Artificial Sequence
  primer 7
gatctgcatgcgatatctctagaacgcgtaagctt

SEQ ID NO: 92 - DNA, 29 bp, Artificial Sequence
  primer 8
tctcgagccgatttattcaacaaagccgc

SEQ ID NO: 93 - DNA, 25 bp, Artificial Sequence
  fw primer
actttcgttttcgggcatttcgtcc

SEQ ID NO: 94 - DNA, 24 bp, Artificial Sequence
  rv primer
ccaatatgagggcagagaacgatc

SEQ ID NO: 95 - DNA, 20 bp, Artificial Sequence
  fw primer
atgcgctgatgtgataatgc

SEQ ID NO: 96 - DNA, 19 bp, Artificial Sequence
  rv primer
ccttctccttgttgcttta

SEQ ID NO: 97 - DNA, 20 bp, Artificial Sequence
  fw primer
gaggcctttgctgcgactgc

SEQ ID NO: 98 - DNA, 21 bp, Artificial Sequence
  rv primer
agttcctccttttcggatgat

SEQ ID NO: 99 - DNA, 18 bp, Artificial Sequence
  fw primer
atgccggatgcgacgctt

SEQ ID NO: 100 - DNA, 20 bp, Artificial Sequence
  rv primer
tcattttgcatatagcccct

SEQ ID NO: 101 - DNA, 20 bp, Artificial Sequence
  fw primer
tgacctgggcagtaatggtg

SEQ ID NO: 102 - DNA, 25 bp, Artificial Sequence
  rv primer
caggatctccgttgctttatgagtc

SEQ ID NO: 103 - DNA, 24 bp, Artificial Sequence
  fw primer
cgtggtgttgaaagccgattattg

SEQ ID NO: 104 - DNA, 23 bp, Artificial Sequence
  rv primer
cataaacttccagttctccgccc

SEQ ID NO: 105 - DNA, 20 bp, Artificial Sequence
  fw primer
tcgcacactaacagactgaa

SEQ ID NO: 106 - DNA, 20 bp, Artificial Sequence
  rv primer
tgtgtttactcctgattagc

SEQ ID NO: 107 - DNA, 25 bp, Artificial Sequence
  fw primer
tattctcaatccgtttcagcacgcg

SEQ ID NO: 108 - DNA, 21 bp, Artificial Sequence
  rv primer
ttcgggatcaccaccaggccg

SEQ ID NO: 109 - DNA, 20 bp, Artificial Sequence
  fw primer
cggaaatggacgaacagtgg

SEQ ID NO: 110 - DNA, 22 bp, Artificial Sequence
  rv primer
cgtcatcagcgtttaccagatt

SEQ ID NO: 111 - DNA, 20 bp, Artificial Sequence
  fw primer
gcataaacactgtccgcgtc

SEQ ID NO: 112 - DNA, 24 bp, Artificial Sequence
  rv primer
gaaatcgagaaggcagaagcgaaa

SEQ ID NO: 113 - DNA, 20 bp, Artificial Sequence
  fw primer
ggtgcggtcaccattgttcg

SEQ ID NO: 114 - DNA, 20 bp, Artificial Sequence
  rv primer
catatcgcacgccagcagtg

SEQ ID NO: 115 - DNA, 21 bp, Artificial Sequence
  fw primer
ggtgaggatggagagttcatg

SEQ ID NO: 116 - DNA, 21 bp, Artificial Sequence
  rv primer
cagttcgatttgcgccaccag

SEQ ID NO: 117 - DNA, 20 bp, Artificial Sequence
  fw primer
tccgctagtgtgatttcagg

SEQ ID NO: 118 - DNA, 23 bp, Artificial Sequence
  rv primer
gaaattattatgccgccaggcgt

SEQ ID NO: 119 - DNA, 20 bp, Artificial Sequence
  fw primer
ttatggtctgggcgacatgc

SEQ ID NO: 120 - DNA, 22 bp, Artificial Sequence
  rv primer
gcatcatcctggtcatataccc

SEQ ID NO: 121 - protein, 455 aa, Natronincola ferrireducens
MLEPKEYIGTLVEKARIAQGEFEKFTQEEVDEVVREMGKVIYDNAVELAKMAVEETRMGIFEDKVKKNQGKSKTIWNSLKGKKSVGIIDRNEETGIVKVAKPVGVVASVTPTTNPIVTPMCNAMFALKGRNAIIIAPHPRAKKCSSYTVELMNKAIAKYRVPENLIQIIEEPSIDLTNELMKAADVVVATGGMGMVQAAYSSGKPAYGVGAGNVQCIVDRDVDIQEVVPKIITGRTFDNGIICSGEQTVIAPEEAYDKIMEEFIKNGGYFVKTPQEKEAFRKALFVDGVISKDVVGQSPQQIAKLAGITIPQDTKVILIEADGIGEEDVLCKEKMCPVLATFKYKDFKDAVTIAQTNLEVEGKGHSCAIHSNNKENIEYAGEKLTISRLVVNQPSSTSAGGSLYNGFAPTTTLGCGTWGNNSISENLNYTHLINVSQIGYFISDRQVPTDEEIWK

SEQ ID NO: 122 - DNA, 28 bp, Artificial Sequence
  fw primer/ I250K
atcaaatgctctggcgaacagagtgtca

SEQ ID NO: 123 - DNA, 28 bp, Artificial Sequence
  fw primer/ I250R
atccgctgctctggcgaacagagtgtca

SEQ ID NO: 124 - DNA, 28 bp, Artificial Sequence
  fw primer/ I250H
atccactgctctggcgaacagagtgtca

SEQ ID NO: 125 - DNA, 28 bp, Artificial Sequence
  fw primer/ I250Q
atcacctgctctggcgaacagagtgtca

SEQ ID NO: 126 - DNA, 28 bp, Artificial Sequence
  fw primer/ I250T
atccagtgctctggcgaacagagtgtca

SEQ ID NO: 127 - DNA, 28 bp, Artificial Sequence
  fw primer/ I250N
atcaactgctctggcgaacagagtgtca

SEQ ID NO: 128 - DNA, 28 bp, Artificial Sequence
  fw primer/ I250G
atcggctgctctggcgaacagagtgtca

SEQ ID NO: 129 - DNA, 28 bp, Artificial Sequence
  fw primer/ I250L
atcgtgtgctctggcgaacagagtgtca

SEQ ID NO: 130 - DNA, 28 bp, Artificial Sequence
  fw primer/ I250V
atcctgtgctctggcgaacagagtgtca

SEQ ID NO: 131 - DNA, 28 bp, Artificial Sequence
  fw primer/ I250W
atctggtgctctggcgaacagagtgtca

SEQ ID NO: 132 - DNA, 28 bp, Artificial Sequence
  fw primer/ I250P
atcccgtgctctggcgaacagagtgtca

SEQ ID NO: 133 - DNA, 34 bp, Artificial Sequence
  rv primer/ I250
cccattatcaaaaatgcgcccggcaataatcttt

SEQ ID NO: 134 - DNA, 33 bp, Artificial Sequence
  fw primer/ F245R
attcgcgataatgggatcatttgctctggcgaa

SEQ ID NO: 135 - DNA, 33 bp, Artificial Sequence
  fw primer/ F245E
attgaagataatgggatcatttgctctggcgaa

SEQ ID NO: 136 - DNA, 33 bp, Artificial Sequence
  fw primer/ F245S
attagcgataatgggatcatttgctctggcgaa

SEQ ID NO: 137 - DNA, 33 bp, Artificial Sequence
  fw primer/ F245N
attaacgataatgggatcatttgctctggcgaa

SEQ ID NO: 138 - DNA, 33 bp, Artificial Sequence
  fw primer/ F245Q
attcaggataatgggatcatttgctctggcgaa

SEQ ID NO: 139 - DNA, 33 bp, Artificial Sequence
  fw primer/ F245G
attggcgataatgggatcatttgctctggcgaa

SEQ ID NO: 140 - DNA, 33 bp, Artificial Sequence
  fw primer/ F245L
attctggataatgggatcatttgctctggcgaa

SEQ ID NO: 141 - DNA, 33 bp, Artificial Sequence
  fw primer/ F245W
atttgggataatgggatcatttgctctggcgaa

SEQ ID NO: 142 - DNA, 25 bp, Artificial Sequence
  rv primer/ F245
gcgcccggcaataatctttggcacc

SEQ ID NO: 143 - DNA, 34 bp, Artificial Sequence
  fw primer/ T405K
gcgaaatctgcaggtggcagctttttcaatggct

SEQ ID NO: 144 - DNA, 34 bp, Artificial Sequence
  fw primer/ T405H
gcgcactctgcaggtggcagctttttcaatggct

SEQ ID NO: 145 - DNA, 34 bp, Artificial Sequence
  fw primer/ T405E
gcggaatctgcaggtggcagctttttcaatggct

SEQ ID NO: 146 - DNA, 34 bp, Artificial Sequence
  fw primer/ T405S
gcgagctctgcaggtggcagctttttcaatggct

SEQ ID NO: 147 - DNA, 34 bp, Artificial Sequence
  fw primer/ T405N
gcgaactctgcaggtggcagctttttcaatggct

SEQ ID NO: 148 - DNA, 34 bp, Artificial Sequence
  fw primer/ T405Q
gcgcagtctgcaggtggcagctttttcaatggct

SEQ ID NO: 149 - DNA, 34 bp, Artificial Sequence
  fw primer/ T405V
gcggtgtctgcaggtggcagctttttcaatggct

SEQ ID NO: 150 - DNA, 34 bp, Artificial Sequence
  fw primer/ T405L
gcgctgtctgcaggtggcagctttttcaatggct

SEQ ID NO: 151 - DNA, 34 bp, Artificial Sequence
  fw primer/ T405Y
gcgtattctgcaggtggcagctttttcaatggct

SEQ ID NO: 152 - DNA, 34 bp, Artificial Sequence
  fw primer/ T405W
gcgtggtctgcaggtggcagctttttcaatggct

SEQ ID NO: 153 - DNA, 34 bp, Artificial Sequence
  fw primer/ T405P
gcgccgtctgcaggtggcagctttttcaatggct

SEQ ID NO: 154 - DNA, 34 bp, Artificial Sequence
  fw primer/ T405F
gcgttttctgcaggtggcagctttttcaatggct

SEQ ID NO: 155 - DNA, 35 bp, Artificial Sequence
  rv primer/ T405
acagcactgattgatcacaaaacgagacacctcaa

SEQ ID NO: 156 - DNA, 28 bp, Artificial Sequence
  fw primer/ T418A
gcgaataccttgggctgtggctcatggg

SEQ ID NO: 157 - DNA, 27 bp, Artificial Sequence
  rv primer/ T418
gggcgctaagccattgaaaaagctgcc